European Patent Application EP 4 393 952 A1, published July 3, 2024. Title: ＣＤ１１６およびＣＤ１３１に結合するバイスペシフィック抗体. Applicant: 協和キリン株式会社. The sequence listing filed with the application follows.

SEQUENCE LISTING (211 sequences)

SEQ ID NO: 1 - DNA, 2691 bp, Homo sapiens
  source 1..2691: mol_type = genomic DNA
atggtgctggctcaaggccttttgagtatggcacttctggccctttgttgggaacggtctctcgccggcgcagaggagacgattccgcttcaaacattgagatgctataacgattatacatctcacattacctgtcggtgggccgacactcaagatgcccagcggcttgtgaacgtaacccttatcagacgggtgaatgaagacctcttggaaccggtatcatgcgatctgtctgacgacatgccgtggagtgcgtgtcctcatccgaggtgcgttccgcggcgctgtgtgatcccgtgtcaaagtttcgtagtgactgatgttgactatttcagtttccagcctgacaggcccctcggaactaggctgaccgtgacgttgactcaacatgtccagcctcctgaacctcgggatttgcagatcagtacagaccaagatcatttccttctgacttggtcagttgctctcggcagtccgcaatcacactggttgtcaccaggtgatctggagttcgaagtagtgtacaagaggcttcaggattcatgggaggatgcagcgatcttgctcagtaatacaagtcaggctacgctcgggccagagcacctcatgccatctagtacttacgtcgcacgcgttcgaactcgcttggcaccgggcagccgacttagcggacggccttccaagtggtccccggaagtatgttgggattctcagccaggggatgaggcccaaccacaaaacttggaatgtttctttgatggtgcggctgttttgagttgtagctgggaagtgcgaaaggaggtggcatccagtgtcagcttcggtctgttctataagccgtctcctgatgcgggtgaggaggagtgtagtccggtcctgcgcgaaggtctgggttccttgcatacccggcaccactgtcaaataccggtccctgacccggctactcacggccagtacatagtatctgtacagccaaggcgggctgagaagcatatcaaaagctcagtgaacattcagatggctcctcccagtttgaatgttaccaaggatggagattcctattcattgaggtgggagaccatgaagatgaggtacgaacacatcgaccatactttcgaaatacaataccgaaaggacactgcgacgtggaaagatagtaaaacggagacgcttcagaacgctcattccatggcgttgcctgctttggagccgtctacgaggtactgggcacgggtaagggtgcggacatctcgcactggctataacgggatatggtcagaatggagtgaagcaagatcatgggataccgagagtgttcttcctatgtgggtgctggccctcatcgtcattttcctcaccatagccgtacttcttgcgctgcgattctgtggaatatacggttatcgcttgagacgcaagtgggaggaaaagattccgaacccttctaagtctcacttgttccagaatggcagtgccgaactttggccgccaggttctatgtcagcattcactagcgggtctccgccccatcagggaccctggggatccagatttccagagctcgaaggcgttttcccggtgggttttggtgactccgaggtatcacctttgacgattgaagatccgaagcacgtttgcgatccacctagtggtcctgacactacgccggccgcatctgatcttccgacagaacaaccaccgtctccacaaccgggaccgccagcagcttcccacacccctgaaaagcaagcttcctctttcgactttaacggtccatatcttggtccaccacactctaggtctctgcccgatatactcggacaacctgagccgcctcaagaaggaggctcacaaaagagcccgcctccagggagtttggaatatctttgcctcccagctggaggtcaagtgcagttggttccccttgcccaggctatggggccaggacaggcagttgaggttgagagacgcccttctcagggtgcagccgggagtccatcacttgagtctggaggagggccagcccctcctgctctcgggccaagagttggtggtcaagatcaaaaggattctccggtagctattccaatgagctctggcgatacagaagaccctggagtcgccagtggttacgtgtcctctgcagacctggtattcactcccaacagtggcgccagttctgtttctctggtaccgagtcttggccttccaagtgatcaaactccgagcctctgcccagggcttgcctcaggtccgccaggagctccaggccctgttaaaagtggcttcgagggttacgttgagctgccgccgatagagggccgcagcccgagatcccctaggaataacccagtacctcccgaagcaaaatcaccagtactcaacccgggcgagcgaccagctgacgtctccccgacaagtccccaacctgaaggcttgttggttctgcaacaagtgggagattactgcttcttgccggggcttggcccggggccattgtctcttaggtctaaaccctccagtcctgggcctggccccgagattaagaatctcgaccaagccttccaagtaaagaagcctccaggtcaagctgttcctcaggtcccagtgatacaacttttcaaggccttgaaacagcaagattacctctccctcccgccttgggaagtcaataagccaggagaagtatgt

SEQ ID NO: 2 - DNA, 2694 bp, Macaca fascicularis
  source 1..2694: mol_type = genomic DNA
atggcattggctcaaaggctgttgtccatggcattgttggccttgtgctggggacactcactgcctggagccgaagaaacaataccactgcgcacgctccgatgctataatgactataccagtcacattacatgtcgctgggcggacactcaagacgcccaaaggttggtcaatgttaccttgagcagacgcgtcaatgatagagaccctccggaacctgtttcttgcgatctctccgaagacatgccgtggtccgcatgcccgtacccgcgatgtgttccacgccgctgtgtcatcccttatcagagctttgtcgtgaccgatgtcgactactactcttttcagccagaccggccccttggtactcaattgacggttacacttacgcaacatgtccaaccgcccgcacctaaggaccttcagatcaatactgatcaggatcacttccttcttacgtggagtgttgcaccaggttcacctcagagccactggctcagccttggtgatcttgagagtgaagtagtgtataagagacttcaagactcttgggaggacgctgctacacttctttccaatgcatctcaggccaccctgggccccgagcatctcatgcccagctctacatacgttgccagagtgaggacccgacttgcaagcgggtctagacttagtggacggccgagcgagtggtctcccgaagtaaggtgggactctcagcctggggatgaagcacagccacaaaaccttcagtgtttcttcgacggggctgctgtgctctcctgcagttgggaagttcggcaagaagtggcatccagtatctcatttgggctcttttacaaaccatctccggacgctggagaggaagaatgcagcccagtgcttagggaaggcctggggtctctttacacaagacaccactgccagattcccgtacccgacccaggcacccacggccagtatattgtcagtgtgcaacctcggagagccgagaaacgcataaagtccagtgaaaatatacaaatggcccccccttctctgtccgttaccagggacggagacagttattctcttcgctgggagacgatgaagatgcagtatgaacacatcgatcatacgttcgaaatacaatatacaaaggacactgctacttggaaggatagcaagacagagactcttcagaacgcacattctatggccctcccggcattggaaccgtccacgcggtactgggcgcgagtccgcgtcagaactagtagaacgggctacaatgggacatggtctgattggagtgaggtctgttcatgggacacggagagcgtacttccgatgtgggtccttgccttggtcgtcatcttcctcaccatagctgtcctgctggccttgcggttctgcggtatttacggatacagactcaggcgaaagtgggaggagcggatacctaacccgtctaagtcacatctgttccagaatggttccgccgagttgtggactccaggttccatgatggcttttacctcaggatcaccacttcaccagggaccatgggacagtagatttcccgagctcgaaggcgtattcccggttgggtttggcgactctgaagtgtccccattgactattgaggatctgcgccacgtctgtgaccctccatccggacccgataccacaccagcggcatccgatctccctacagaacaacctccgtccccacagccgggacctccagcctccagtcatacgcccgagaagcaagtttcaagctttgatttcaacgggccctacttgggccctccgcactcccggtcactgccagacatcctgggtcagccagaaccgcctcaagcttgcgggtcccagaagagcccgcctccgggtagtctcgaatacctctgcctgcccgcaggcggccaagttcaattggtccctctggctcaggctatgggacacggtcaagcgatggacgttgaacggcggccgtctcaaggagccgcaggatcctccagtcttgaatctgagggcgacccggcgccaccggccttgggaccacgcgttggcggacaagacccgaaggacagtcctgtagcaattccggcctccagcggggtcccggaggacccaggggtcgcatcaggttacgtatcctctgctgacttggtactgccaccccactcaggcacgtctgctctttcactcgtgccatccccgggaatcccttcagatcaaacaccctctttctgcccgggtttggcaagtggaccaccaggcgctccaggtcctgttaagtccgaatttgagggatatgtggaactgccgccgacagaaggacagagtcctaagtctcctgtgaacaacttggtgccaccggaagtacggtcccctgttcttaaccccggcgagagacgggccgacgtgagtcctaccagcccgcaacccgaggggctcttggtgctccaacaagttggggattactgcttccttccggggctcggtcctggccctctgagtccccggtcaaaaccgtctagtcctggcccgtgccctgaaatcagagacctcgaccaggcctgtcaggtgaagaaaccgccggggcaggcggtccctcaggtgccggtcattcaactgttcaaggtactcaaacaacaggattacctgtcccttcctccgtgggaggttaacaagccaggcgaagtgtgt

SEQ ID NO: 3 - DNA, 1281 bp, Homo sapiens
  source 1..1281: mol_type = genomic DNA
tgggaacggagtctggccggagctgaggagacaattccactgcagacattgcgctgctacaatgactatacctcccacatcacatgtcggtgggctgacacgcaagacgcccagagactggtgaatgtgactctgattcggcgagtgaatgaggatctcttggagcccgtttcttgcgatctgagcgacgacatgccttggagcgcatgtccccatcctaggtgcgtgcccaggaggtgcgtaataccctgtcagagctttgtggtgacagacgtggactacttctccttccagccggataggcctctgggcactagattgaccgttactctcactcagcacgtacaaccgccggaacccagggacctccaaatctccacagaccaggatcacttcctcctgacctggtcagtagctctgggcagtccacagtctcactggcttagccctggggatttggagtttgaagtcgtgtacaaacgtctgcaggatagctgggaggatgccgcgattctgctgagcaacacttcccaagcaacacttggcccagagcacctgatgccttccagcacctatgtcgctagagtccgcactaggcttgcaccaggaagccggttgtcaggtcgcccctctaaatggtccccagaggtctgttgggactcacaacctggggacgaagcccagccgcagaaccttgagtgcttctttgatggtgccgcagtgctctcatgtagttgggaagtcagaaaagaggttgccagcagcgtgtcctttggcctgttctataagccatcacccgatgccggggaagaagagtgctctcctgtactgagggaaggactcggatctctccatacccgacaccattgccagataccagtgcctgatccagccactcatggccagtacatcgttagtgtgcaaccccgcagagctgagaagcacatcaagagcagtgtcaacattcagatggcacctccctctctgaacgtgaccaaagatggtgacagctactcccttcggtgggaaacgatgaagatgcgttatgaacacatcgatcacacctttgagatccagtaccgcaaggatacggccacatggaaggacagcaaaaccgaaacactgcagaatgcgcactcaatggcactgccagctctggaaccctccacccggtattgggcccgagttcgtgtgcgcacctccagaacaggctacaacgggatttggagtgagtggtcagaggcgagatcttgggacaccgagtctgtcctgcccatgtgg

SEQ ID NO: 4 - DNA, 873 bp, Macaca fascicularis
  source 1..873: mol_type = genomic DNA
gagaaaccagcaagctctctgaatgtccggtttgatgcgaggaccatgaatctcacatgggattgccaggaaaacaccacctttacccgctgttttctgactgacaagaagaatagagttgtagagcccagagtgactaagaaagaatgctcctgtacgttccacgaggtttgcctgcacggaggtgtgacattcgaggttcacgtgaatactagtcaaagggcatttcagcagaagctgctgtatcccaattctgggagagaagggacagccgctcagaacttctcctgcttcatctacaacgtggatttcatgaactgtacctgggctagaggtccaactgctcctcgggatgtgcagtacttcctgtacatacagaacagcaaacgtcgcagggagatccaatgcccctactacatcgaggactcaggcacacatgtgggatgtcacctcggcaatcttagcggccttactagccgaaactactttctggtcaatgggacctctcaggagattgggattcagttctttgattccctcctggacacgaagaagatagagaggttcaatcctcctggcaatgtcacggtacggtgcaacacaacccactgtttggttcggtggaaacaaccgaggacctatcagaaactctcatatctggacttccagtatcagcttgacgtgcatcggaagaatacccaaccaggcacagaaaatctgcctatcaacgtgtctggagacttggagaaccgctataactttcccagcagtgaaccacgagccaagcatgccgtcaaaattagagctgccgatgtgcgtatcctgaactggtccagctggtcagaagcagccgaatttggaagtgatgaccgc

SEQ ID NO: 5 - DNA, 1257 bp, Mus musculus
  source 1..1257: mol_type = genomic DNA
catggggtgactgaggctgaagaaaccgttcccctgaaaacgctgcaatgctacaacgattataccaaccacatcatttgcagctgggcagataccgaggacgcccaaggattgatcaacatgacgctgtaccatcagctggagaagaaacagcctgtctcctgtgagctctccgaagaactgatgtggtcagaatgtcccagtagccataggtgtgttccccggcgttgcgtgattccctacacaaggttcagtatcaccaatgaggactactacagctttagaccagactcagatctcggcatacaactgatggtacctctggctcagaatgtgcagccacccttgcctaagaatgtcagcatttccagcagcgaagatcgcttcctcttggaatggtccgtgtcacttggtgatgcccaagtgtcttggttgagttccaaggacatcgagtttgaggtcgcctataagcggctgcaggatagctgggaggacgcgtatagccttcacacatctaagtttcaggtgaacttcgagccaaagctgttcctgcccaattccatctatgcagcacgcgttcggacacgactgtctccaggatcatccctctccgggcgaccttctagatggtcaccggaagtgcactgggactcacagcctggagataaagcacagccacagaaccttcagtgcttctttgacgggatccaatcccttcactgctcatgggaggtgtggactcaaaccaccggcagtgtgagctttggcctcttttacaggccctctcctgtggctccggaagagaaatgttctcccgtagtaaaagagcctccgggagctagcgtctatacccgttatcactgcagtctgcctgttcctgaaccctccgctcactctcagtacacagtgagtgtcaaacacctggaacagggtaagttcatcatgagctataaccacattcagatggaaccaccaacactcaacctcactaagaatcgcgactcctattccctgcattgggagactcagaaaatggcctacagtttcattgagcacactttccaggtccagtacaagaagaagagcgactcatgggaggactctaaaactgagaatctggatagagcccatagtatggatctgagccagctggaaccagataccagctattgtgccagggttagagtgaagccaatcagcaactacgacggcatatggtctaagtggtctgaggagtacacatggaaaacagactgg

SEQ ID NO: 6 - DNA, 1200 bp, Homo sapiens
  source 1..1200: mol_type = genomic DNA
atgctgcttcttgtgacctctcttctgctgtgcgaactgccccatcctgcctttctgctgattcccgagaaatccgacttgaggacagtagccccagcatctagtctgaacgtgagattcgatagtcgaactatgaacctgtcatgggactgtcaggagaacactaccttcagcaagtgctttctgactgacaagaagaacagggttgtggaaccgagactgagcaataacgaatgctcttgtacattccgggagatttgcctgcatgagggagttaccttcgaagtgcacgtgaacacgagccaacgcggtttccagcagaaactgctgtaccccaactcagggagagaaggaacagcagcccagaactttagctgcttcatctacaatgccgatctcatgaactgtacctgggctagaggccctacagctccacgcgacgttcagtacttcctctacattcggaatagcaaacgtcgtcgcgagatacgatgtccctattacatccaggattctggcacacatgtgggttgccatttggacaatctgtcaggcttgacatcccggaactatttcctggtgaacggcactagccgcgaaattggcatccagttcttcgacagccttcttgataccaagaaaattgagcgatttaaccctccctccaatgtgacagtacgctgtaataccactcactgtctggtgcgctggaagcagcccagaacctatcagaagctctcttatctggactttcagtatcaactggatgtccacagaaagaacacccaacctggcactgagaatttgctgatcaatgtcagtggtgatttggagaatcggtacaactttccatcctcagaaccaagggcgaaacactccgtgaagatcagggctgcagatgttaggatcctgaattggagcagttggtctgaagccatagagtttgggtccgatgacgggaatctgggaagcgtctacatctacgtgctcctcattgtcgggaccttggtatgcggaattgtcctcggattcctctttaaacggttcctgagaatacaaaggctgtttccacctgtgccgcagatcaaggataagctcaatgacaatcacgaagtggaggacgagattatctgggaggagtttactcctgaggaagggaaaggctatcgggaggaagtccttacggttaaagagatcacg

SEQ ID NO: 7 - DNA, 1179 bp, Macaca fascicularis
  source 1..1179: mol_type = genomic DNA
atgtttctgctggtgacctctcttgtactgtttgaactgctgcaaccagcgtttctgctgatacccgagaaaccagcctctagcctgaatgtgcgctttgacgctagaacgatgaatctcacatgggactgccaggaaaacaccacatttagccgatgtttcctcactgacaagaaaggccgtgttgtcgagccaagggtaaccaacaaggagtgttcctgcacctttagggaaatttgcttgcatggaggcgtcacgttcgaagtgcacgtgaatacttcccaaagaacctttcaggagaagctgctgtatcccaactctggaagggaagggacagcagcccagaactttagctgcttcatctacaatgtggactttatgaactgtacttgggcacgtggtcctactgctcctcgcgatgtgcagtatttcctgtatatccagaacagcaaacggaggcgagagattcagtgcccatactacattgaggattcagggacacacgttggctgtcacctgggtaatcttagcggtctgacctcacgaaactacttcctcgttaacggcacatctcaagagataggcattcagttcttcgattccttgctcgacaccaagaaaatcgagcgcttcaatcctccagggaatgtcacagtgcgctgcaatactacccactgtctggtgagatggaaacaacctcggacctatcagaaactgagctacctggatttccagtatcagcttgacgtacaccggaagaatatgcaacccggaacggaaaaccttcccatcaacgtgagtggagatctggagaatcggtacaactttcccagttccgaaccgagagcgaagcatgccgtcaagatcagagctgccgatgtgcggatactgaactggagttcctggtctgaagcagccgagtttgggtcagatgacaggaaccccagttcagtgcatatctatgtgctcctgatactgggtacactggtctgtgttctcttgttcggctttctctttaagcgtttctttcgaatccagaggcttttcccgccagttccccagatcaaagacaaactgaatgacaaccacgaggttgaggacgaaatcatttgggaggagttcatgccagaagagggcaagggctatcgcgaagaagtcctgactgtcaaagaaatcacg

SEQ ID NO: 8 - DNA, 894 bp, Homo sapiens
  source 1..894: mol_type = genomic DNA
gagaaatccgacttgcgaactgtcgcaccagccagctctctgaatgtccgatttgactctcggacaatgaacctgagttgggactgtcaggagaataccaccttcagcaaatgcttcctgactgataagaagaatcgggtggttgaacctagactctccaacaatgagtgctcatgtacctttagggagatatgcctgcatgaaggtgtgacgttcgaagtgcacgtgaacacctcccaaaggggctttcagcagaagctgctgtatcccaatagcgggagagagggcactgctgcgcagaatttcagctgcttcatctacaacgctgatctgatgaactgcacatgggcaagaggccctacagccccgagagatgtgcagtacttcctctacataaggaactccaaaagacgcagggaaattcggtgtccctattacatccaggatagcggaactcacgtgggatgtcaccttgacaatctgtcagggcttacaagtcgcaactattttctcgtcaatgggacatctcgcgagattggcatccaattctttgactcactgctggacaccaagaaaatcgagcgtttcaatccacccagtaacgtgacggtacgctgcaacaccacacactgtttggtcaggtggaaacagcctcgtacctaccagaaactctcctatttggacttccagtatcagcttgatgtacaccgaaagaacactcaaccaggtaccgagaatctgctgatcaacgtttccggagatctggaaaaccggtacaactttccctcatctgaacctagagccaagcatagcgtgaagattcgcgcagctgacgttcggattctcaattggagctcttggagcgaagccatcgagtttggcagtgatgacgga

SEQ ID NO: 9 - DNA, 891 bp, Macaca fascicularis
  source 1..891: mol_type = genomic DNA
gagaaaccagcctctagcctgaatgtgcgctttgacgctagaacgatgaatctcacatgggactgccaggaaaacaccacatttagccgatgtttcctcactgacaagaaaggccgtgttgtcgagccaagggtaaccaacaaggagtgttcctgcacctttagggaaatttgcttgcatggaggcgtcacgttcgaagtgcacgtgaatacttcccaaagaacctttcaggagaagctgctgtatcccaactctggaagggaagggacagcagcccagaactttagctgcttcatctacaatgtggactttatgaactgtacttgggcacgtggtcctactgctcctcgcgatgtgcagtatttcctgtatatccagaacagcaaacggaggcgagagattcagtgcccatactacattgaggattcagggacacacgttggctgtcacctgggtaatcttagcggtctgacctcacgaaactacttcctcgttaacggcacatctcaagagataggcattcagttcttcgattccttgctcgacaccaagaaaatcgagcgcttcaatcctccagggaatgtcacagtgcgctgcaatactacccactgtctggtgagatggaaacaacctcggacctatcagaaactgagctacctggatttccagtatcagcttgacgtacaccggaagaatatgcaacccggaacggaaaaccttcccatcaacgtgagtggagatctggagaatcggtacaactttcccagttccgaaccgagagcgaagcatgccgtcaagatcagagctgccgatgtgcggatactgaactggagttcctggtctgaagcagccgagtttgggtcagatgacaggcatcaccaccatcatcac

SEQ ID NO: 10 - DNA, 894 bp, Mus musculus
  source 1..894: mol_type = genomic DNA
cttttggcccctaccacacctgatgccggctcagccctcaacctgacattcgatccttggacaaggaccctcacatgggcctgtgatacagcagctgggaatgtgacggtaaccagctgcaccgtgactagtcgggaagcaggaatccatcgaagggttagtccctttgggtgtcggtgctggttcagacggatgatggccttgcatcacggtgtgactctggatgtgaatggcaccgtaggaggagcagctgcccattggcggttgagcttcgtcaacgaaggggcagctggttctggcgcagagaatctgacgtgcgagataagggcagcacggtttctgtcctgtgcctggcgagagggacccgctgccccagccgatgttcgctactccctcagggttctcaactctacaggtcacgacgtcgccagatgtatggctgatccaggggatgacgtcattacgcagtgcatcgcgaacgaccttagccttctgggcagtgaggcctatctggtggtgactggccgttcaggagcaggacccgtcagatttctggacgacgttgtggccactaaagcgctggaacgactcggccctccacgcgacgtgactgcttcctgcaactcctctcactgtaccgtgagctgggctccaccctcaacctgggctagcctgactgcgcgtgacttccagttcgaggtgcagtggcaatccgctgagccggggagcacaccccgcaaggtactggtcgttgaggaaaccagactggcctttccctctcctgcaccgcatggtggccacaaggtcaaagtgagggctggggacacacgcatgaagcactggggcgaatggagtccagctcatcctctggaagccgaggacaccagagtgcca

SEQ ID NO: 11 - protein, 123 aa, Homo sapiens
EVQLVESGGGLVKPGGSLRLSCVASELTFSNVWMTWVRQAPGKGLEWVGRIKSKADGGTTDYAAPVKGRFTISRDDSKNTLYLQMNSLKTEDTAVYYCTTGGYSYGDNWFDPWGQGTLVTVSS

SEQ ID NO: 12 - protein, 107 aa, Homo sapiens
EIVLTQSPATLSLSPGERATLSCRASQSVSSYLAWYQQKPGQAPRLLIYDASNRATGIPARFSGSGSGTDFTLTISSLEPEDFAVYYCQQRSNWPWTFGQGTKVEIK

SEQ ID NO: 13 - protein, 126 aa, Homo sapiens
EVQLVESGGGLVQPGRSLRLSCAASGFTFDDYAMHWVRQAPGKGLEWVSGISWNSGIIGYADSVKGRFTISRDNAKNSLYLQMNSLRAEDTALYYCAKDTGSSGWYDYNYYGMDVWGQGTTVTVSS

SEQ ID NO: 14 - protein, 107 aa, Homo sapiens
AIQLTQSPSSLSASVGDRVTITCRASQGISSVLAWYQQKPGKAPKLLIYDASSLESGVPSRFSGSGSGTDFTLTISSLQPEDFATYYCQQFNSYPRTFGQGTKVEIK

SEQ ID NO: 15 - protein, 126 aa, Homo sapiens
EVQLVESGGGLVQPGRSLRLSCAASGFTFGDYAMHWVRQAPGKGLEWVSGISWNSGIIGYADSVKGRFTISRDNAKNSLYLQMNSLRAEDTALYYCVKDEGSSGWYDFNYFGMDVWGQGTTVTVSS

SEQ ID NO: 16 - protein, 107 aa, Homo sapiens
AIQLTQSPSSLSASVGDRVTITCRASQGISSALAWYQQKPGKAPKLLIYDASSLESGVPSRFSGSGSGTDFTLTISSLQPEDFATYYCQQFNSYPITFGQGTRLEIK

SEQ ID NO: 17 - protein, 126 aa, Homo sapiens
EVQLVESGGGLVQPGRSLRLSCAASGFTFDDYAMHWVRQAPGKGLEWVSGISWNSGIIGYADSVKGRFTISRDNAKNSLYLQMNSLRAEDTALYYCAKDMGSSGWYDYNYFGMDVWGQGTTVTVSS

SEQ ID NO: 18 - protein, 107 aa, Homo sapiens; identical to SEQ ID NO: 14

SEQ ID NO: 19 - protein, 114 aa, Homo sapiens
QVQLVQSGAEVKKPGASVKVSCKVSGYTLTEFSIHWVRQAPGKGLEWMGGFDPEDDETIYAQKFQGRVTMTEDTSTDTAYMELSSLRSEDTAVYYCATSQMLLWGQGTMVTVSS

SEQ ID NO: 20 - protein, 107 aa, Homo sapiens
DIQMTQSPSSLSASVGDRVTITCRASQGISSWLAWYQQKPEKAPKSLIYAASSLQSGVPSRFSGSGSGTDFTLTISSLQPEDFATYYCQQYNSYPHTFGQGTKLEIK

SEQ ID NO: 21 - protein, 122 aa, Homo sapiens
EVQLVESGGGLVKPGGSLRLSCEASGFTLSSYTMNWVRQAPGKGLEWVSSIRSSSSFIYYADSVKGRFTISRDIAKNSLYLQINSLRAEDTAVYYCARDYYGSGSYWYFDLWGRGTLVTVSS

SEQ ID NO: 22 - protein, 107 aa, Homo sapiens
EIVLTQSPATLSLSPGERATLSCRASQSVSSYLAWYQQKPGQAPRLLIYDASNRATGIPARFSGSGSGTDFTLTISSLEPEDFAVYYCQQRSNWPLTFGGGTKVEIK

SEQ ID NO: 23 - protein, 124 aa, Homo sapiens
QVQLVESGGGLVKPGGSLRLSCAASGFTFSDYYMSWIRQAPGKGLEWVSFISSSGIIIYYADSVKGRFTISRDNAKNSLYLQMNSLRAEDTAVYYCARRGYSGYDYYYYGLDVWGQGTTVTVSS

SEQ ID NO: 24 - protein, 105 aa, Homo sapiens
EIVLTQSPGTLSLSPGERATLSCRASQSVSSSYLAWYQQKPGQAPRLLIYGASSRATGIPDRFSGSGSGTDFTLTISRLEPEDFAVYYCQQYGSTFGGGTKVEIK

SEQ ID NO: 25 - protein, 118 aa, Homo sapiens
QVQLVESGGGLVKPGGSLRLSCAASGFTFSDYYMNWIRQAPGKGLEWVSYISTSGSIIYYADSVKGRFTISRDNAKNSLYLQMNSLRAEDTAVYYCARRRYYYGMDVWGQGTTVTVSS

SEQ ID NO: 26 - protein, 105 aa, Homo sapiens
EIVLTQSPGTLSLSPGERATLSCRASQSVSSSYLAWYQQKPGQAPRLLIYGASSRATGIPDRFSGSGSGTDFTLTISRLEPEDFAVYYCQQYGRTFGQGTKVEIK

SEQ ID NO: 27 - protein, 128 aa, Homo sapiens
QVQLVQSGAEVKKPGASVKVSCKASGYTFTSDYMHWVRQAPGQGLEWMGIINPSGGATSYVQKFQGRVTMTRDTSTSTVYMELSSLRSEDTAVYYCARERYYGSGTYFNIGLWYFDLWGRGTLVTVSS

SEQ ID NO: 28 - protein, 108 aa, Homo sapiens
EIVLTQSPGTLSLSPGERATLSCRASQSVSSSYLAWYQQKPGQAPRLLIYGASSRATGIPDRFSGSGSGTDFTLTISRLEPEDFAVYYCQQYGSSPLTFGGGTKVEIK

SEQ ID NO: 29 - protein, 128 aa, Homo sapiens
QVQLVQSGAEVKEPGASVKISCKASGYTFTNDYMHWVRQAPGQGLEWMGIINPTGGGTSYAQKFRGRVTMTRDTSTSTVYMELSSLRSEDTAVFYCARERYYGSGTYFNIGLWYFDLWGRGTLVTVSS

SEQ ID NO: 30 - protein, 108 aa, Homo sapiens; identical to SEQ ID NO: 28

SEQ ID NO: 31 - protein, 5 aa, Homo sapiens
NVWMT

SEQ ID NO: 32 - protein, 19 aa, Homo sapiens
RIKSKADGGTTDYAAPVKG

SEQ ID NO: 33 - protein, 12 aa, Homo sapiens
GGYSYGDNWFDP

SEQ ID NO: 34 - protein, 11 aa, Homo sapiens
RASQSVSSYLA

SEQ ID NO: 35 - protein, 7 aa, Homo sapiens
DASNRAT

SEQ ID NO: 36 - protein, 9 aa, Homo sapiens
QQRSNWPWT

SEQ ID NO: 37 - protein, 5 aa, Homo sapiens
DYAMH

SEQ ID NO: 38 - protein, 17 aa, Homo sapiens
GISWNSGIIGYADSVKG

SEQ ID NO: 39 - protein, 17 aa, Homo sapiens
DTGSSGWYDYNYYGMDV

SEQ ID NO: 40 - protein, 11 aa, Homo sapiens
RASQGISSVLA

SEQ ID NO: 41 - protein, 7 aa, Homo sapiens
DASSLES

SEQ ID NO: 42 - protein, 9 aa, Homo sapiens
QQFNSYPRT

SEQ ID NO: 43 - protein, 5 aa, Homo sapiens
DYAMH

SEQ ID NO: 44 - protein, 17 aa, Homo sapiens
GISWNSGIIGYADSVKG

SEQ ID NO: 45 - protein, 17 aa, Homo sapiens
DEGSSGWYDFNYFGMDV

SEQ ID NO: 46 - protein, 11 aa, Homo sapiens
RASQGISSALA

SEQ ID NO: 47 - protein, 7 aa, Homo sapiens
DASSLES

SEQ ID NO: 48 - protein, 9 aa, Homo sapiens
QQFNSYPIT

SEQ ID NO: 49 - protein, 5 aa, Homo sapiens
DYAMH

SEQ ID NO: 50 - protein, 17 aa, Homo sapiens
GISWNSGIIGYADSVKG

SEQ ID NO: 51 - protein, 17 aa, Homo sapiens
DMGSSGWYDYNYFGMDV

SEQ ID NO: 52 - protein, 11 aa, Homo sapiens
RASQGISSVLA

SEQ ID NO: 53 - protein, 7 aa, Homo sapiens
DASSLES

SEQ ID NO: 54 - protein, 9 aa, Homo sapiens
QQFNSYPRT

SEQ ID NO: 55 - protein, 5 aa, Homo sapiens
EFSIH

SEQ ID NO: 56 - protein, 17 aa, Homo sapiens
GFDPEDDETIYAQKFQG

SEQ ID NO: 57 - protein, 5 aa, Homo sapiens
SQMLL

SEQ ID NO: 58 - protein, 11 aa, Homo sapiens
RASQGISSWLA

SEQ ID NO: 59 - protein, 7 aa, Homo sapiens
AASSLQS

SEQ ID NO: 60 - protein, 9 aa, Homo sapiens
QQYNSYPHT

SEQ ID NO: 61 - protein, 5 aa, Homo sapiens
SYTMN

SEQ ID NO: 62 - protein, 17 aa, Homo sapiens
SIRSSSSFIYYADSVKG

SEQ ID NO: 63 - protein, 13 aa, Homo sapiens
DYYGSGSYWYFDL

SEQ ID NO: 64 - protein, 11 aa, Homo sapiens
RASQSVSSYLA

SEQ ID NO: 65 - protein, 7 aa, Homo sapiens
DASNRAT

SEQ ID NO: 66 - protein, 9 aa, Homo sapiens
QQRSNWPLT

SEQ ID NO: 67 - protein, 5 aa, Homo sapiens
DYYMS

SEQ ID NO: 68 - protein, 17 aa, Homo sapiens
FISSSGIIIYYADSVKG

SEQ ID NO: 69 - protein, 15 aa, Homo sapiens
RGYSGYDYYYYGLDV

SEQ ID NO: 70 - protein, 12 aa, Homo sapiens
RASQSVSSSYLA

SEQ ID NO: 71 - protein, 7 aa, Homo sapiens
GASSRAT

SEQ ID NO: 72 - protein, 6 aa, Homo sapiens
QQYGST

SEQ ID NO: 73 - protein, 5 aa, Homo sapiens
DYYMN

SEQ ID NO: 74 - protein, 17 aa, Homo sapiens
YISTSGSIIYYADSVKG

SEQ ID NO: 75 - protein, 9 aa, Homo sapiens
RRYYYGMDV

SEQ ID NO: 76 - protein, 12 aa, Homo sapiens
RASQSVSSSYLA

SEQ ID NO: 77 - protein, 7 aa, Homo sapiens
GASSRAT

SEQ ID NO: 78 - protein, 6 aa, Homo sapiens
QQYGRT

SEQ ID NO: 79 - protein, 5 aa, Homo sapiens
SDYMH

SEQ ID NO: 80 - protein, 17 aa, Homo sapiens
IINPSGGATSYVQKFQG

SEQ ID NO: 81 - protein, 19 aa, Homo sapiens
ERYYGSGTYFNIGLWYFDL

SEQ ID NO: 82 - protein, 12 aa, Homo sapiens
RASQSVSSSYLA

SEQ ID NO: 83 - protein, 7 aa, Homo sapiens
GASSRAT

SEQ ID NO: 84 - protein, 9 aa, Homo sapiens
QQYGSSPLT

SEQ ID NO: 85 - protein, 5 aa, Homo sapiens
NDYMH

SEQ ID NO: 86 - protein, 17 aa, Homo sapiens
IINPTGGGTSYAQKFRG

SEQ ID NO: 87 - protein, 19 aa, Homo sapiens
ERYYGSGTYFNIGLWYFDL

SEQ ID NO: 88 - protein, 12 aa, Homo sapiens
RASQSVSSSYLA

SEQ ID NO: 89 - protein, 7 aa, Homo sapiens
GASSRAT

SEQ ID NO: 90 - protein, 9 aa, Homo sapiens
QQYGSSPLT

SEQ ID NO: 91 - protein, 324 aa, Homo sapiens
GAAATTGTGTTGACGCAGTCTCCAGGCACCCTGTCTTTGTCTCCAGGGGAAAGAGCCACCCTCTCCTGCAGGGCCAGTCAGAGTGTTAGCAGCAGCTACTTAGCCTGGTACCAGCAGAAACCTGGCCAGGCTCCCAGGCTCCTCATCTATGGTGCATCCAGCAGGGCCACTGGCATCCCAGACAGGTTCAGTGGCAGTGGGTCTGGGACAGACTTCACTCTCACCATCAGCAGACTGGAGCCTGAAGATTTTGCAGTGTATTACTGTCAGCAGTATGGTAGCTCACCGCTCACTTTCGGCGGAGGGACCAAGGTGGAGATCAAA

SEQ ID NO: 92 - protein, 120 aa, Homo sapiens
EVQLVQSGAEVKKPGASVKVSCKVSGYTLAELSMHWVRQAPGKGLEWMGGFDPEDGERIYAQKFQGRVTMTEDTSKDTAYMELSSLRSEDTAVYYCTTGLFYYQYGMDVWGQGTMVTVSS

SEQ ID NO: 93 - protein, 120 aa, Homo sapiens
EVQLVQSGAEVKKPGASVKVSCKVSGYTLTDLSMHWVRQAPGKGLEWMGGLDPEDGETIYAQKFQGRVTMTEDTSTDTAYMELSSLRSEDTAVYYCATGLFYYQYGMDVWGQGTLVTVSS

SEQ ID NO: 94 - protein, 120 aa, Homo sapiens
QVQLVQSGAEVKKPGASVKVSCKVSGYTLTDLSMHWVRQAPGKGLEWMGGFDPEDGETIYAQKFQGRVTMTEDTSTDTAYMELSSLRSEDTAVYYCATGLFYYQYGMDVWGQGTTVTVSS

SEQ ID NO: 95 - protein, 120 aa, Homo sapiens
QVQLQQSGAEVKKPGASVKVSCKVSGYTLTDLSMHWVRQAPGKGLEWMGGFDPEDGERIYAQKFQGRVTMTEDTATDTAYMELSSLRSEDTAVYHCATGLFYYQYGMDVWGQGTTVTVSS

SEQ ID NO: 96 - protein, 120 aa, Homo sapiens
QVQLVQSGAEVKKPGASVKVSCKVSGYTLTDFAIHWVRQAPGKGLEWMGGFDPEDGERIYAQKFQGRVTMTEDTSTDTAYMELSSLRSEDTAVYYCTTGLFYYQYGMDVWGQGTLVTVSS

SEQ ID NO: 97 - protein, 120 aa, Homo sapiens
EVQLVQSGAEVKKPGASVKVSCKVSGYTLTELSMHWVRQAPGKGLEWMGGFDPEDGERIYAQKFQGRVTMTEDTSTDTAYMELSSLRSEDTAVYYCATGLFYYQYGMDVWGQGTTVTVSS

SEQ ID NO: 98 - protein, 120 aa, Homo sapiens
QVQLQQSGAEVKKPGASVKVSCKVSGYTLTDLSMHWVRQAPGKGLEWMGGFDPEDGERIYAQKFQGRVTMTEDTSTDTAYMELSSLRSEDTAVYYCATGLFYYQYGMDVWGQGTLVTVSS

SEQ ID NO: 99 - protein, 120 aa, Homo sapiens
QVQLVQSGAEVKKPGASVKVSCKVSGYTLTDFAIHWVRQAPGKGLEWMGGFDPEDGERIYAQKFQGRVTMTEDTSTDTAYMELSSLRSEDTAVYYCATGLFYYQYGMDVWGQGTTVTVSS

SEQ ID NO: 100 - protein, 120 aa, Homo sapiens
QVQLVQSGAEVKKPGASVKVSCKVSGYTLTDLSMHWVRQAPGKGLEWMGGFDPEDGERIYAQKFQGRVTMTEDTSTDTAYMELSSLRSEDTAMYYCATGLFYYQYGMDVWGQGTTVTVSS

SEQ ID NO: 101 - protein, 120 aa, Homo sapiens
QVQLVQSGAEVKKPGASVKVSCKVSGYPLTDLSMHWVRQAPGEGLEWMGGSDPEDGETIYAQKFQGRVTVTEDTSTDTAYMELSNLRSEDTAVYYCATGLFYYQYGMDVWGQGTTVTVSS

SEQ ID NO: 102 - protein, 120 aa, Homo sapiens
QVQLVQSGAEVKKPGASVKVSCKVSGYTLTDLSMHWVRQAPGKGLEWMGGFDPEDGERIYAQKFQDRVTMTEDTSTDTAYMELSSLRSEDTAVYYCATGLFYYQYGMDVWGQGTLVTVSS

SEQ ID NO: 103 - protein, 120 aa, Homo sapiens
EVQLVQSGAEVKKPGASVKVSCKVSGYTLTDLSMHWVRQAPGKGLEWMGGFDPEDGERIYAQKFQGRVTMTEDTSTDTAYMELSSLRSEDTAVYYCATGLFYYYYGMDVWGQGTMVTVSS

SEQ ID NO: 104 - protein, 5 aa, Homo sapiens
ELSMH

SEQ ID NO: 105 - protein, 17 aa, Homo sapiens
GFDPEDGERIYAQKFQG

SEQ ID NO: 106 - protein, 11 aa, Homo sapiens
GLFYYQYGMDV

SEQ ID NO: 107 - protein, 5 aa, Homo sapiens
DLSMH

SEQ ID NO: 108 - protein, 17 aa, Homo sapiens
GLDPEDGETIYAQKFQG

SEQ ID NO: 109 - protein, 11 aa, Homo sapiens
GLFYYQYGMDV

SEQ ID NO: 110 - protein, 5 aa, Homo sapiens
DLSMH

SEQ ID NO: 111 - protein, 17 aa, Homo sapiens
GFDPEDGETIYAQKFQG

SEQ ID NO: 112 - protein, 11 aa, Homo sapiens
GLFYYQYGMDV

SEQ ID NO: 113 - protein, 5 aa, Homo sapiens
DLSMH

SEQ ID NO: 114 - protein, 17 aa, Homo sapiens
GFDPEDGERIYAQKFQG

SEQ ID NO: 115 - protein, 11 aa, Homo sapiens
GLFYYQYGMDV

SEQ ID NO: 116 - protein, 5 aa, Homo sapiens
DFAIH

SEQ ID NO: 117 - protein, 17 aa, Homo sapiens
GFDPEDGERIYAQKFQG

SEQ ID NO: 118 - protein, 11 aa, Homo sapiens
GLFYYQYGMDV

SEQ ID NO: 119 - protein, 5 aa, Homo sapiens
ELSMH

SEQ ID NO: 120 - protein, 17 aa, Homo sapiens
GFDPEDGERIYAQKFQG

SEQ ID NO: 121 - protein, 11 aa, Homo sapiens
GLFYYQYGMDV

SEQ ID NO: 122 - protein, 5 aa, Homo sapiens
DLSMH

SEQ ID NO: 123 - protein, 17 aa, Homo sapiens
GFDPEDGERIYAQKFQG

SEQ ID NO: 124 - protein, 11 aa, Homo sapiens
GLFYYQYGMDV

SEQ ID NO: 125 - protein, 5 aa, Homo sapiens
DFAIH

SEQ ID NO: 126 - protein, 17 aa, Homo sapiens
GFDPEDGERIYAQKFQG

SEQ ID NO: 127 - protein, 11 aa, Homo sapiens
GLFYYQYGMDV

SEQ ID NO: 128 - protein, 5 aa, Homo sapiens
DLSMH

SEQ ID NO: 129 - protein, 17 aa, Homo sapiens
GFDPEDGERIYAQKFQG

SEQ ID NO: 130 - protein, 11 aa, Homo sapiens
GLFYYQYGMDV

SEQ ID NO: 131 - protein, 5 aa, Homo sapiens
DLSMH

SEQ ID NO: 132 - protein, 17 aa, Homo sapiens
GSDPEDGETIYAQKFQG

SEQ ID NO: 133 - protein, 11 aa, Homo sapiens
GLFYYQYGMDV

SEQ ID NO: 134 - protein, 5 aa, Homo sapiens
DLSMH

SEQ ID NO: 135 - protein, 17 aa, Homo sapiens
GFDPEDGERIYAQKFQD

SEQ ID NO: 136 - protein, 11 aa, Homo sapiens
GLFYYQYGMDV

SEQ ID NO: 137 - protein, 5 aa, Homo sapiens
DLSMH

SEQ ID NO: 138 - protein, 17 aa, Homo sapiens
GFDPEDGERIYAQKFQG

SEQ ID NO: 139 - protein, 11 aa, Homo sapiens
GLFYYYYGMDV

SEQ ID NO: 140 - protein, 330 aa, Homo sapiens
ASTKGPSVCPLAPSSKSTSGGTAALGCLVKDYFPEPVTVSWNSGALTSGVHTFPAVLQSSGLYSLSSVVTVPSSSLGTQTYICNVNHKPSNTKVDKKVEPKSADKTHTCPPCPAPEAAGGPSVFLFPPKPKDTLMISRTPEVTCVVVDVSHEDPEVKFNWYVDGVEVHNAKTKPREEQYNSTYRVVSVLTVLHQDWLNGKEYKCKVSNKALGAPIEKTISKAKGQPREPQVYTLPPCRDELTKNQVSLWCLVKGFYPSDIAVEWESNGQPENNYKTTPPVLDSDGSFFLYSKLTVDKSRWQQGNVFSCSVMHEALHNHYTQKSLSLSPGK

SEQ ID NO: 141 - protein, 107 aa, Homo sapiens
RTVAAPSVFIFPPCDEQLKSGTASVVCLLNNFYPREAKVQWKVDNALQSGNSQESVTEQDSKDSTYSLSSTLTLSKADYEKHKVYACEVTHQGLSSPVTKSFNRGES

SEQ ID NO: 142 - protein, 330 aa, Homo sapiens
ASTKGPSVFPLAPSSKSTSGGTAALGCLVKDYFPEPVTVSWNSGALTSGVHTFPAVLQSSGLYSLSSVVTVPSSSLGTQTYICNVNHKPSNTKVDKKVEPKSCDKTHTCPPCPAPEAAGGPSVFLFPPKPKDTLMISRTPEVTCVVVDVSHEDPEVKFNWYVDGVEVHNAKTKPREEQYNSTYRVVSVLTVLHQDWLNGKEYKCKVSNKALGAPIEKTISKAKGQPREPQVCTLPPSRDELTKNQVSLSCAVKGFYPSDIAVEWESNGQPENNYKTTPPVLDSDGSFFLVSKLTVDKSRWQQGNVFSCSVMHEALHNRFTQKSLSLSPGK

SEQ ID NO: 143 - protein, 107 aa, Homo sapiens [sequence omitted]

SEQ ID NO: 144 - protein, 98 aa, Homo sapiens
ASTKGPSVFPLAPCSRSTSESTAALGCLVKDYFPEPVTVSWNSGALTSGVHTFPAVLQSSGLYSLSSVVTVPSSSLGTKTYTCNVDHKPSNTKVDKRV

SEQ ID NO: 145 - protein, 327 aa, Homo sapiens
ASTKGPSVFPLAPCSRSTSESTAALGCLVKDYFPEPVTVSWNSGALTSGVHTFPAVLQSSGLYSLSSVVTVPSSSLGTKTYTCNVDHKPSNTKVDKRVESKYGPPCPPCPAPEFEGGPSVFLFPPKPKDTLMISRTPEVTCVVVDVSQEDPEVQFNWYVDGVEVHNAKTKPREEQFNSTYRVVSVLTVLHQDWLNGKEYKCKVSNKGLPSSIEKTISKAKGQPREPQVYTLPPSQEEMTKNQVSLTCLVKGFYPSDIAVEWESNGQPENNYKTTPPVLDSDGSFFLYSKLTVDKSRWQEGNVFSCSVMHEALHNHYTQKSLSLSLGK

SEQ ID NO: 146 - protein, 330 aa, Homo sapiens
ASTKGPSVFPLAPSSKSTSGGTAALGCLVKDYFPEPVTVSWNSGALTSGVHTFPAVLQSSGLYSLSSVVTVPSSSLGTQTYICNVNHKPSNTKVDKKVEPKSCDKTHTCPPCPAPEAAGAPSVFLFPPKPKDTLMISRTPEVTCVVVDVSHEDPEVKFNWYVDGVEVHNAKTKPREEQYNSTYRVVSVLTVLHQDWLNGKEYKCKVSNKALPAPIEKTISKAKGQPREPQVYTLPPSRDELTKNQVSLTCLVKGFYPSDIAVEWESNGQPENNYKTTPPVLDSDGSFFLYSKLTVDKSRWQQGNVFSCSVMHEALHNHYTQKSLSLSPGK

SEQ ID NO: 147 - protein, 327 aa, Homo sapiens
ASTKGPSVFPLAPCSRSTSESTAALGCLVKDYFPEPVTVSWNSGALTSGVHTFPAVLQSSGLYSLSSVVTVPSSSLGTKTYTCNVDHKPSNTKVDKRVESKYGPPCPPCPAPEFEGGPSVFLFPPKPKDTLMASRTPEVTCVVVDVSQEDPEVQFNWYVDGVEVHNAKTKPREEQFNSTYRVVSVLTVLHQDWLNGKEYKCKVSNKGLPSSIEKTISKAKGQPREPQVYTLPPSQEEMTKNQVSLTCLVKGFYPSDIAVEWESNGQPENNYKTTPPVLDSDGSFFLYSKLTVDKSRWQEGNVFSCSVMHEALHNHYTQKSLSLSLGK

SEQ ID NO: 148 - protein, 327 aa, Homo sapiens
ASTKGPSVFPLAPCSRSTSESTAALGCLVKDYFPEPVTVSWNSGALTSGVHTFPAVLQSSGLYSLSSVVTVPSSSLGTKTYTCNVDHKPSNTKVDKRVESKYGPPCPPCPAPEFEGGPSVFLFPPKPKDTLMHSRTPEVTCVVVDVSQEDPEVQFNWYVDGVEVHNAKTKPREEQFNSTYRVVSVLTVLHQDWLNGKEYKCKVSNKGLPSSIEKTISKAKGQPREPQVYTLPPSQEEMTKNQVSLTCLVKGFYPSDIAVEWESNGQPENNYKTTPPVLDSDGSFFLYSKLTVDKSRWQEGNVFSCSVMHEALHNHYTQKSLSLSLGK

SEQ ID NO: 149 - protein, 327 aa, Homo sapiens
ASTKGPSVFPLAPCSRSTSESTAALGCLVKDYFPEPVTVSWNSGALTSGVHTFPAVLQSSGLYSLSSVVTVPSSSLGTKTYTCNVDHKPSNTKVDKRVESKYGPPCPPCPAPEFEGGPSVFLFPPKPKDTLMDSRTPEVTCVVVDVSQEDPEVQFNWYVDGVEVHNAKTKPREEQFNSTYRVVSVLTVLHQDWLNGKEYKCKVSNKGLPSSIEKTISKAKGQPREPQVYTLPPSQEEMTKNQVSLTCLVKGFYPSDIAVEWESNGQPENNYKTTPPVLDSDGSFFLYSKLTVDKSRWQEGNVFSCSVMHEALHNHYTQKSLSLSLGK

SEQ ID NO: 150 - protein, 327 aa, Homo sapiens
ASTKGPSVFPLAPCSRSTSESTAALGCLVKDYFPEPVTVSWNSGALTSGVHTFPAVLQSSGLYSLSSVVTVPSSSLGTKTYTCNVDHKPSNTKVDKRVESKYGPPCPPCPAPEFEGGPSVFLFPPKPKDTLMSSRTPEVTCVVVDVSQEDPEVQFNWYVDGVEVHNAKTKPREEQFNSTYRVVSVLTVLHQDWLNGKEYKCKVSNKGLPSSIEKTISKAKGQPREPQVYTLPPSQEEMTKNQVSLTCLVKGFYPSDIAVEWESNGQPENNYKTTPPVLDSDGSFFLYSKLTVDKSRWQEGNVFSCSVMHEALHNHYTQKSLSLSLGK

SEQ ID NO: 151 - protein, 327 aa, Homo sapiens
ASTKGPSVFPLAPCSRSTSESTAALGCLVKDYFPEPVTVSWNSGALTSGVHTFPAVLQSSGLYSLSSVVTVPSSSLGTKTYTCNVDHKPSNTKVDKRVESKYGPPCPPCPAPEFEGGPSVFLFPPKPKDTLMISRTPEVTCVVVDVSQEDPEVQFNWYVDGVEVHNAKTKPREEQFNSTYRVVSVLTVLDQDWLNGKEYKCKVSNKGLPSSIEKTISKAKGQPREPQVYTLPPSQEEMTKNQVSLTCLVKGFYPSDIAVEWESNGQPENNYKTTPPVLDSDGSFFLYSKLTVDKSRWQEGNVFSCSVMHEALHNHYTQKSLSLSLGK

SEQ ID NO: 152 - protein, 327 aa, Homo sapiens
ASTKGPSVFPLAPCSRSTSESTAALGCLVKDYFPEPVTVSWNSGALTSGVHTFPAVLQSSGLYSLSSVVTVPSSSLGTKTYTCNVDHKPSNTKVDKRVESKYGPPCPPCPAPEFEGGPSVFLFPPKPKDTLMISRTPEVTCVVVDVSQEDPEVQFNWYVDGVEVHNAKTKPREEQFNSTYRVVSVLTVLGQDWLNGKEYKCKVSNKGLPSSIEKTISKAKGQPREPQVYTLPPSQEEMTKNQVSLTCLVKGFYPSDIAVEWESNGQPENNYKTTPPVLDSDGSFFLYSKLTVDKSRWQEGNVFSCSVMHEALHNHYTQKSLSLSLGK

SEQ ID NO: 153 - protein, 327 aa, Homo sapiens
ASTKGPSVFPLAPCSRSTSESTAALGCLVKDYFPEPVTVSWNSGALTSGVHTFPAVLQSSGLYSLSSVVTVPSSSLGTKTYTCNVDHKPSNTKVDKRVESKYGPPCPPCPAPEFEGGPSVFLFPPKPKDTLMISRTPEVTCVVVDVSQEDPEVQFNWYVDGVEVHNAKTKPREEQFNSTYRVVSVLTVLHQDWLNGKEYKCKVSNKGLPSSIEKTISKAKGQPREPQVYTLPPSQEEMTKNQVSLTCLVKGFYPSDIAVEWESNGQPENNYKTTPPVLDSDGSFFLYSKLTVDKSRWQEGNVFSCSVMHEALHNAYTQKSLSLSLGK

SEQ ID NO: 154 - protein, 327 aa, Homo sapiens
ASTKGPSVFPLAPCSRSTSESTAALGCLVKDYFPEPVTVSWNSGALTSGVHTFPAVLQSSGLYSLSSVVTVPSSSLGTKTYTCNVDHKPSNTKVDKRVESKYGPPCPPCPAPEFEGGPSVFLFPPKPKDTLMISRTPEVTCVVVDVSQEDPEVQFNWYVDGVEVHNAKTKPREEQFNSTYRVVSVLTVLHQDWLNGKEYKCKVSNKGLPSSIEKTISKAKGQPREPQVYTLPPSQEEMTKNQVSLTCLVKGFYPSDIAVEWESNGQPENNYKTTPPVLDSDGSFFLYSKLTVDKSRWQEGNVFSCSVMHEALHNEYTQKSLSLSLGK

SEQ ID NO: 155 - protein, 327 aa, Homo sapiens
ASTKGPSVFPLAPCSRSTSESTAALGCLVKDYFPEPVTVSWNSGALTSGVHTFPAVLQSSGLYSLSSVVTVPSSSLGTKTYTCNVDHKPSNTKVDKRVESKYGPPCPPCPAPEFEGGPSVFLFPPKPKDTLMISRTPEVTCVVVDVSQEDPEVQFNWYVDGVEVHNAKTKPREEQFNSTYRVVSVLTVLHQDWLNGKEYKCKVSNKGLPSSIEKTISKAKGQPREPQVYTLPPSQEEMTKNQVSLTCLVKGFYPSDIAVEWESNGQPENNYKTTPPVLDSDGSFFLYSKLTVDKSRWQEGNVFSCSVMHEALHNFYTQKSLSLSLGK

SEQ ID NO: 156 - protein, 327 aa, Homo sapiens
ASTKGPSVFPLAPCSRSTSESTAALGCLVKDYFPEPVTVSWNSGALTSGVHTFPAVLQSSGLYSLSSVVTVPSSSLGTKTYTCNVDHKPSNTKVDKRVESKYGPPCPPCPAPEFEGGPSVFLFPPKPKDTLMISRTPEVTCVVVDVSQEDPEVQFNWYVDGVEVHNAKTKPREEQFNSTYRVVSVLTVLHQDWLNGKEYKCKVSNKGLPSSIEKTISKAKGQPREPQVYTLPPSQEEMTKNQVSLTCLVKGFYPSDIAVEWESNGQPENNYKTTPPVLDSDGSFFLYSKLTVDKSRWQEGNVFSCSVMHEALHNTYTQKSLSLSLGK

SEQ ID NO: 157 - protein, 327 aa, Homo sapiens
ASTKGPSVFPLAPCSRSTSESTAALGCLVKDYFPEPVTVSWNSGALTSGVHTFPAVLQSSGLYSLSSVVTVPSSSLGTKTYTCNVDHKPSNTKVDKRVESKYGPPCPPCPAPEFEGGPSVFLFPPKPKDTLMISRTPEVTCVVVDVSQEDPEVQFNWYVDGVEVHNAKTKPREEQFNSTYRVVSVLTVLHQDWLNGKEYKCKVSNKGLPSSIEKTISKAKGQPREPQVYTLPPSQEEMTKNQVSLTCLVKGFYPSDIAVEWESNGQPENNYKTTPPVLDSDGSFFLYSKLTVDKSRWQEGNVFSCSVMHEALHNHATQKSLSLSLGK

SEQ ID NO: 158 - protein, 327 aa, Homo sapiens
ASTKGPSVFPLAPCSRSTSESTAALGCLVKDYFPEPVTVSWNSGALTSGVHTFPAVLQSSGLYSLSSVVTVPSSSLGTKTYTCNVDHKPSNTKVDKRVESKYGPPCPPCPAPEFEGGPSVFLFPPKPKDTLMISRTPEVTCVVVDVSQEDPEVQFNWYVDGVEVHNAKTKPREEQFNSTYRVVSVLTVLHQDWLNGKEYKCKVSNKGLPSSIEKTISKAKGQPREPQVYTLPPSQEEMTKNQVSLTCLVKGFYPSDIAVEWESNGQPENNYKTTPPVLDSDGSFFLYSKLTVDKSRWQEGNVFSCSVMHEALHNHETQKSLSLSLGK

SEQ ID NO: 159 - protein, 327 aa, Homo sapiens
ASTKGPSVFPLAPCSRSTSESTAALGCLVKDYFPEPVTVSWNSGALTSGVHTFPAVLQSSGLYSLSSVVTVPSSSLGTKTYTCNVDHKPSNTKVDKRVESKYGPPCPPCPAPEFEGGPSVFLFPPKPKDTLMISRTPEVTCVVVDVSQEDPEVQFNWYVDGVEVHNAKTKPREEQFNSTYRVVSVLTVLHQDWLNGKEYKCKVSNKGLPSSIEKTISKAKGQPREPQVYTLPPSQEEMTKNQVSLTCLVKGFYPSDIAVEWESNGQPENNYKTTPPVLDSDGSFFLYSKLTVDKSRWQEGNVFSCSVMHEALHNHGTQKSLSLSLGK

SEQ ID NO: 160 - protein, 330 aa, Homo sapiens
ASTKGPSVFPLAPSSKSTSGGTAALGCLVKDYFPEPVTVSWNSGALTSGVHTFPAVLQSSGLYSLSSVVTVPSSSLGTQTYICNVNHKPSNTKVDKKVEPKSCDKTHTCPPCPAPEAAGAPSVFLFPPKPKDTLMASRTPEVTCVVVDVSHEDPEVKFNWYVDGVEVHNAKTKPREEQYNSTYRVVSVLTVLHQDWLNGKEYKCKVSNKALPAPIEKTISKAKGQPREPQVYTLPPSRDELTKNQVSLTCLVKGFYPSDIAVEWESNGQPENNYKTTPPVLDSDGSFFLYSKLTVDKSRWQQGNVFSCSVMHEALHNHYTQKSLSLSPGK

SEQ ID NO: 161 - protein, 330 aa, Homo sapiens
ASTKGPSVFPLAPSSKSTSGGTAALGCLVKDYFPEPVTVSWNSGALTSGVHTFPAVLQSSGLYSLSSVVTVPSSSLGTQTYICNVNHKPSNTKVDKKVEPKSCDKTHTCPPCPAPEAAGAPSVFLFPPKPKDTLMHSRTPEVTCVVVDVSHEDPEVKFNWYVDGVEVHNAKTKPREEQYNSTYRVVSVLTVLHQDWLNGKEYKCKVSNKALPAPIEKTISKAKGQPREPQVYTLPPSRDELTKNQVSLTCLVKGFYPSDIAVEWESNGQPENNYKTTPPVLDSDGSFFLYSKLTVDKSRWQQGNVFSCSVMHEALHNHYTQKSLSLSPGK

SEQ ID NO: 162 - protein, 330 aa, Homo sapiens
ASTKGPSVFPLAPSSKSTSGGTAALGCLVKDYFPEPVTVSWNSGALTSGVHTFPAVLQSSGLYSLSSVVTVPSSSLGTQTYICNVNHKPSNTKVDKKVEPKSCDKTHTCPPCPAPEAAGAPSVFLFPPKPKDTLMDSRTPEVTCVVVDVSHEDPEVKFNWYVDGVEVHNAKTKPREEQYNSTYRVVSVLTVLHQDWLNGKEYKCKVSNKALPAPIEKTISKAKGQPREPQVYTLPPSRDELTKNQVSLTCLVKGFYPSDIAVEWESNGQPENNYKTTPPVLDSDGSFFLYSKLTVDKSRWQQGNVFSCSVMHEALHNHYTQKSLSLSPGK

SEQ ID NO: 163 - protein, 330 aa, Homo sapiens
ASTKGPSVFPLAPSSKSTSGGTAALGCLVKDYFPEPVTVSWNSGALTSGVHTFPAVLQSSGLYSLSSVVTVPSSSLGTQTYICNVNHKPSNTKVDKKVEPKSCDKTHTCPPCPAPEAAGAPSVFLFPPKPKDTLMSSRTPEVTCVVVDVSHEDPEVKFNWYVDGVEVHNAKTKPREEQYNSTYRVVSVLTVLHQDWLNGKEYKCKVSNKALPAPIEKTISKAKGQPREPQVYTLPPSRDELTKNQVSLTCLVKGFYPSDIAVEWESNGQPENNYKTTPPVLDSDGSFFLYSKLTVDKSRWQQGNVFSCSVMHEALHNHYTQKSLSLSPGK

SEQ ID NO: 164 - protein, 330 aa, Homo sapiens
ASTKGPSVFPLAPSSKSTSGGTAALGCLVKDYFPEPVTVSWNSGALTSGVHTFPAVLQSSGLYSLSSVVTVPSSSLGTQTYICNVNHKPSNTKVDKKVEPKSCDKTHTCPPCPAPEAAGAPSVFLFPPKPKDTLMISRTPEVTCVVVDVSHEDPEVKFNWYVDGVEVHNAKTKPREEQYNSTYRVVSVLTVLDQDWLNGKEYKCKVSNKALPAPIEKTISKAKGQPREPQVYTLPPSRDELTKNQVSLTCLVKGFYPSDIAVEWESNGQPENNYKTTPPVLDSDGSFFLYSKLTVDKSRWQQGNVFSCSVMHEALHNHYTQKSLSLSPGK

SEQ ID NO: 165 - protein, 330 aa, Homo sapiens
ASTKGPSVFPLAPSSKSTSGGTAALGCLVKDYFPEPVTVSWNSGALTSGVHTFPAVLQSSGLYSLSSVVTVPSSSLGTQTYICNVNHKPSNTKVDKKVEPKSCDKTHTCPPCPAPEAAGAPSVFLFPPKPKDTLMISRTPEVTCVVVDVSHEDPEVKFNWYVDGVEVHNAKTKPREEQYNSTYRVVSVLTVLGQDWLNGKEYKCKVSNKALPAPIEKTISKAKGQPREPQVYTLPPSRDELTKNQVSLTCLVKGFYPSDIAVEWESNGQPENNYKTTPPVLDSDGSFFLYSKLTVDKSRWQQGNVFSCSVMHEALHNHYTQKSLSLSPGK

SEQ ID NO: 166 - protein, 330 aa, Homo sapiens
ASTKGPSVFPLAPSSKSTSGGTAALGCLVKDYFPEPVTVSWNSGALTSGVHTFPAVLQSSGLYSLSSVVTVPSSSLGTQTYICNVNHKPSNTKVDKKVEPKSCDKTHTCPPCPAPEAAGAPSVFLFPPKPKDTLMISRTPEVTCVVVDVSHEDPEVKFNWYVDGVEVHNAKTKPREEQYNSTYRVVSVLTVLHQDWLNGKEYKCKVSNKALPAPIEKTISKAKGQPREPQVYTLPPSRDELTKNQVSLTCLVKGFYPSDIAVEWESNGQPENNYKTTPPVLDSDGSFFLYSKLTVDKSRWQQGNVFSCSVMHEALHNAYTQKSLSLSPGK

SEQ ID NO: 167 - protein, 330 aa, Homo sapiens
ASTKGPSVFPLAPSSKSTSGGTAALGCLVKDYFPEPVTVSWNSGALTSGVHTFPAVLQSSGLYSLSSVVTVPSSSLGTQTYICNVNHKPSNTKVDKKVEPKSCDKTHTCPPCPAPEAAGAPSVFLFPPKPKDTLMISRTPEVTCVVVDVSHEDPEVKFNWYVDGVEVHNAKTKPREEQYNSTYRVVSVLTVLHQDWLNGKEYKCKVSNKALPAPIEKTISKAKGQPREPQVYTLPPSRDELTKNQVSLTCLVKGFYPSDIAVEWESNGQPENNYKTTPPVLDSDGSFFLYSKLTVDKSRWQQGNVFSCSVMHEALHNEYTQKSLSLSPGK

SEQ ID NO: 168 - protein, 330 aa, Homo sapiens
ASTKGPSVFPLAPSSKSTSGGTAALGCLVKDYFPEPVTVSWNSGALTSGVHTFPAVLQSSGLYSLSSVVTVPSSSLGTQTYICNVNHKPSNTKVDKKVEPKSCDKTHTCPPCPAPEAAGAPSVFLFPPKPKDTLMISRTPEVTCVVVDVSHEDPEVKFNWYVDGVEVHNAKTKPREEQYNSTYRVVSVLTVLHQDWLNGKEYKCKVSNKALPAPIEKTISKAKGQPREPQVYTLPPSRDELTKNQVSLTCLVKGFYPSDIAVEWESNGQPENNYKTTPPVLDSDGSFFLYSKLTVDKSRWQQGNVFSCSVMHEALHNFYTQKSLSLSPGK

SEQ ID NO: 169 - protein, 330 aa, Homo sapiens
ASTKGPSVFPLAPSSKSTSGGTAALGCLVKDYFPEPVTVSWNSGALTSGVHTFPAVLQSSGLYSLSSVVTVPSSSLGTQTYICNVNHKPSNTKVDKKVEPKSCDKTHTCPPCPAPEAAGAPSVFLFPPKPKDTLMISRTPEVTCVVVDVSHEDPEVKFNWYVDGVEVHNAKTKPREEQYNSTYRVVSVLTVLHQDWLNGKEYKCKVSNKALPAPIEKTISKAKGQPREPQVYTLPPSRDELTKNQVSLTCLVKGFYPSDIAVEWESNGQPENNYKTTPPVLDSDGSFFLYSKLTVDKSRWQQGNVFSCSVMHEALHNTYTQKSLSLSPGK

SEQ ID NO: 170 - protein, 330 aa, Homo sapiens
ASTKGPSVFPLAPSSKSTSGGTAALGCLVKDYFPEPVTVSWNSGALTSGVHTFPAVLQSSGLYSLSSVVTVPSSSLGTQTYICNVNHKPSNTKVDKKVEPKSCDKTHTCPPCPAPEAAGAPSVFLFPPKPKDTLMISRTPEVTCVVVDVSHEDPEVKFNWYVDGVEVHNAKTKPREEQYNSTYRVVSVLTVLHQDWLNGKEYKCKVSNKALPAPIEKTISKAKGQPREPQVYTLPPSRDELTKNQVSLTCLVKGFYPSDIAVEWESNGQPENNYKTTPPVLDSDGSFFLYSKLTVDKSRWQQGNVFSCSVMHEALHNHATQKSLSLSPGK

SEQ ID NO: 171 - protein, 330 aa, Homo sapiens
ASTKGPSVFPLAPSSKSTSGGTAALGCLVKDYFPEPVTVSWNSGALTSGVHTFPAVLQSSGLYSLSSVVTVPSSSLGTQTYICNVNHKPSNTKVDKKVEPKSCDKTHTCPPCPAPEAAGAPSVFLFPPKPKDTLMISRTPEVTCVVVDVSHEDPEVKFNWYVDGVEVHNAKTKPREEQYNSTYRVVSVLTVLHQDWLNGKEYKCKVSNKALPAPIEKTISKAKGQPREPQVYTLPPSRDELTKNQVSLTCLVKGFYPSDIAVEWESNGQPENNYKTTPPVLDSDGSFFLYSKLTVDKSRWQQGNVFSCSVMHEALHNHETQKSLSLSPGK

SEQ ID NO: 172 - protein, 330 aa, Homo sapiens
ASTKGPSVFPLAPSSKSTSGGTAALGCLVKDYFPEPVTVSWNSGALTSGVHTFPAVLQSSGLYSLSSVVTVPSSSLGTQTYICNVNHKPSNTKVDKKVEPKSCDKTHTCPPCPAPEAAGAPSVFLFPPKPKDTLMISRTPEVTCVVVDVSHEDPEVKFNWYVDGVEVHNAKTKPREEQYNSTYRVVSVLTVLHQDWLNGKEYKCKVSNKALPAPIEKTISKAKGQPREPQVYTLPPSRDELTKNQVSLTCLVKGFYPSDIAVEWESNGQPENNYKTTPPVLDSDGSFFLYSKLTVDKSRWQQGNVFSCSVMHEALHNHGTQKSLSLSPGK

SEQ ID NO: 173 - DNA, 384 bp, Homo sapiens
  source 1..384: mol_type = genomic DNA
caggtgcagctcgtgcagtccggagccgaagtgaaggagccaggagcctccgtgaagatctcctgcaaggcctccggctacaccttcaccaacgactacatgcactgggtgaggcaggccccaggacagggactggagtggatggggatcatcaaccccacaggaggagggacatcctatgcccagaagttccgcggacgcgtgacaatgacacgcgacacatccacatccacagtgtacatggagctgtcctccctgcgctccgaggacacagccgtgttctactgtgcccgcgaacgctactatggctccgggacctacttcaacatcgggctgtggtacttcgacctgtggggacgcggaacactcgtgacagtgtcctcc

SEQ ID NO: 174 - DNA, 294 bp, Homo sapiens
  source 1..294: mol_type = genomic DNA
gcgtccacaaaggggccctccgtgttcccgctggccccatgttcccgctccacatccgagtccacagctgccctgggatgtctcgtgaaggattactttcccgagcccgtgacagtgtcctggaactccggggccctgacatccggcgtccacacattcccagccgtgctgcagtcctccgggctgtactccctgtcctccgtcgtgacagtgccatcctcctccctggggaccaagacatacacatgcaacgtggaccacaagccctccaacacaaaagtggacaagcgcgtg

SEQ ID NO: 175 - protein, 120 aa, Homo sapiens; identical to SEQ ID NO: 92

SEQ ID NO: 176 - protein, 120 aa, Homo sapiens
EVQLQESGAEVKKPGASVKVSCKVSGYTLTDLSMHWVRQAPGKGLEWMGGLDPEDGETIYAQKFQGRVTMTEDTSTDTAYMELSSLRSEDTAVYYCATGLFYYQYGMDVWGQGTLVTVSS

SEQ ID NO: 177 - protein, 120 aa, Homo sapiens
EVQLEQSGAEVKKPGASVKVSCKVSGYTLTDLSMHWVRQAPGKGLEWMGGFDPEDGETIYAQKFQGRVTMTEDTSTDTAYMELSSLRSEDTAVYYCATGLFYYQYGMDVWGQGTTVTVSS

SEQ ID NO: 178 - protein, 120 aa, Homo sapiens
EVQLVESGAEVKKPGASVKVSCKVSGYTLTDLSMHWVRQAPGKGLEWMGGFDPEDGERIYAQKFQGRVTMTEDTATDTAYMELSSLRSEDTAVYHCATGLFYYQYGMDVWGQGTTVTVSS

SEQ ID NO: 179 - protein, 120 aa, Homo sapiens
QVQLVESGAEVKKPGASVKVSCKVSGYTLTDFAIHWVRQAPGKGLEWMGGFDPEDGERIYAQKFQGRVTMTEDTSTDTAYMELSSLRSEDTAVYYCTTGLFYYQYGMDVWGQGTLVTVSS

SEQ ID NO: 180 - protein, 120 aa, Homo sapiens; identical to SEQ ID NO: 97

SEQ ID NO: 181 - protein, 120 aa, Homo sapiens; identical to SEQ ID NO: 98

SEQ ID NO: 182 - protein, 120 aa, Homo sapiens
EVQLVQSGAEVKKPGASVKVSCKVSGYTLTDFAIHWVRQAPGKGLEWMGGFDPEDGERIYAQKFQGRVTMTEDTSTDTAYMELSSLRSEDTAVYYCATGLFYYQYGMDVWGQGTTVTVSS

SEQ ID NO: 183 - protein, 120 aa, Homo sapiens
EVQLLQSGAEVKKPGASVKVSCKVSGYTLTDLSMHWVRQAPGKGLEWMGGFDPEDGERIYAQKFQGRVTMTEDTSTDTAYMELSSLRSEDTAMYYCATGLFYYQYGMDVWGQGTTVTVSS

SEQ ID NO: 184 - protein, 120 aa, Homo sapiens
QVQLQESGAEVKKPGASVKVSCKVSGYPLTDLSMHWVRQAPGEGLEWMGGSDPEDGETIYAQKFQGRVTVTEDTSTDTAYMELSNLRSEDTAVYYCATGLFYYQYGMDVWGQGTTVTVSS

SEQ ID NO: 185 - protein, 120 aa, Homo sapiens
EVQLVQSGAEVKKPGASVKVSCKVSGYTLTDLSMHWVRQAPGKGLEWMGGFDPEDGERIYAQKFQDRVTMTEDTSTDTAYMELSSLRSEDTAVYYCATGLFYYQYGMDVWGQGTLVTVSS

SEQ ID NO: 186 - protein, 120 aa, Homo sapiens; identical to SEQ ID NO: 103

SEQ ID NO: 187 - protein, 1579 aa, Homo sapiens
MLLLVTSLLLCELPHPAFLLIPEKSDLRTVAPASSLNVRFDSRTMNLSWDCQENTTFSKCFLTDKKNRVVEPRLSNNECSCTFREICLHEGVTFEVHVNTSQRGFQQKLLYPNSGREGTAAQNFSCFIYNADLMNCTWARGPTAPRDVQYFLYIRNSKRRREIRCPYYIQDSGTHVGCHLDNLSGLTSRNYFLVNGTSREIGIQFFDSLLDTKKIERFNPPSNVTVRCNTTHCLVRWKQPRTYQKLSYLDFQYQLDVHRKNTQPGTENLLINVSGDLENRYNFPSSEPRAKHSVKIRAADVRILNWSSWSEAIEFGSDDGNLGSVYIYVLLIVGTLVCGIVLGFLFKRFLRIQRLFPPVPQIKDKLNDNHEVEDEIIWEEFTPEEGKGYREEVLTVKEITRAKRAPVKQTLNFDLLKLAGDVESNPGPMVLAQGLLSMALLALCWERSLAGAEETIPLQTLRCYNDYTSHITCRWADTQDAQRLVNVTLIRRVNEDLLEPVSCDLSDDMPWSACPHPRCVPRRCVIPCQSFVVTDVDYFSFQPDRPLGTRLTVTLTQHVQPPEPRDLQISTDQDHFLLTWSVALGSPQSHWLSPGDLEFEVVYKRLQDSWEDAAILLSNTSQATLGPEHLMPSSTYVARVRTRLAPGSRLSGRPSKWSPEVCWDSQPGDEAQPQNLECFFDGAAVLSCSWEVRKEVASSVSFGLFYKPSPDAGEEECSPVLREGLGSLHTRHHCQIPVPDPATHGQYIVSVQPRRAEKHIKSSVNIQMAPPSLNVTKDGDSYSLRWETMKMRYEHIDHTFEIQYRKDTATWKDSKTETLQNAHSMALPALEPSTRYWARVRVRTSRTGYNGIWSEWSEARSWDTESVLPMWVLALIVIFLTIAVLLALRFCGIYGYRLRRKWEEKIPNPSKSHLFQNGSAELWPPGSMSAFTSGSPPHQGPWGSRFPELEGVFPVGFGDSEVSPLTIEDPKHVCDPPSGPDTTPAASDLPTEQPPSPQPGPPAASHTPEKQASSFDFNGPYLGPPHSRSLPDILGQPEPPQEGGSQKSPPPGSLEYLCLPAGGQVQLVPLAQAMGPGQAVEVERRPSQGAAGSPSLESGGGPAPPALGPRVGGQDQKDSPVAIPMSSGDTEDPGVASGYVSSADLVFTPNSGASSVSLVPSLGLPSDQTPSLCPGLASGPPGAPGPVKSGFEGYVELPPIEGRSPRSPRNNPVPPEAKSPVLNPGERPADVSPTSPQPEGLLVLQQVGDYCFLPGLGPGPLSLRSKPSSPGPGPEIKNLDQAFQVKKPPGQAVPQVPVIQLFKALKQQDYLSLPPWEVNKPGEVCRAKRAPVKQTLNFDLLKLAGDVESNPGPMVSVIKPEMKIKLCMRGTVNGHNFVIEGEGKGNPYEGTQILDLNVTEGAPLPFAYDILTTVFQYGNRAFTKYPADIQDYFKQTFPEGYHWERSMTYEDQGICTATSNISMRGDCFFYDIRFDGTNFPPNGPVMQKKTLKWEPSTEKMYVEDGVLKGDVNMRLLLEGGGHYRCDFKTTYKAKKEVRLPDAHKIDHRIEILKHDKDYNKVKLYENAVARYSMLPSQAK

SEQ ID NO: 188 - protein, 1557 aa, Homo sapiens
MVLLWLTLLLIALPCLLQTKEDPNPPITNLRMKAKAQQLTWDLNRNVTDIECVKDADYSMPAVNNSYCQFGAISLCEVTNYTVRVANPPFSTWILFPENSGKPWAGAENLTCWIHDVDFLSCSWAVGPGAPADVQYDLYLNVANRRQQYECLHYKTDAQGTRIGCRFDDISRLSSGSQSSHILVRGRSAAFGIPCTDKFVVFSQIEILTPPNMTAKCNKTHSFMHWKMRSHFNRKFRYELQIQKRMQPVITEQVRDRTSFQLLNPGTYTVQIRARERVYEFLSAWSTPQRFECDQEEGANTRAWRTSLLIALGTLLALVCVFVICRRYLVMQRLFPRIPHMKDPIGDSFQNDKLVVWEAGKAGLEECLVTEVQVVQKTRAKRAPVKQTLNFDLLKLAGDVESNPGPMVLAQGLLSMALLALCWERSLAGAEETIPLQTLRCYNDYTSHITCRWADTQDAQRLVNVTLIRRVNEDLLEPVSCDLSDDMPWSACPHPRCVPRRCVIPCQSFVVTDVDYFSFQPDRPLGTRLTVTLTQHVQPPEPRDLQISTDQDHFLLTWSVALGSPQSHWLSPGDLEFEVVYKRLQDSWEDAAILLSNTSQATLGPEHLMPSSTYVARVRTRLAPGSRLSGRPSKWSPEVCWDSQPGDEAQPQNLECFFDGAAVLSCSWEVRKEVASSVSFGLFYKPSPDAGEEECSPVLREGLGSLHTRHHCQIPVPDPATHGQYIVSVQPRRAEKHIKSSVNIQMAPPSLNVTKDGDSYSLRWETMKMRYEHIDHTFEIQYRKDTATWKDSKTETLQNAHSMALPALEPSTRYWARVRVRTSRTGYNGIWSEWSEARSWDTESVLPMWVLALIVIFLTIAVLLALRFCGIYGYRLRRKWEEKIPNPSKSHLFQNGSAELWPPGSMSAFTSGSPPHQGPWGSRFPELEGVFPVGFGDSEVSPLTIEDPKHVCDPPSGPDTTPAASDLPTEQPPSPQPGPPAASHTPEKQASSFDFNGPYLGPPHSRSLPDILGQPEPPQEGGSQKSPPPGSLEYLCLPAGGQVQLVPLAQAMGPGQAVEVERRPSQGAAGSPSLESGGGPAPPALGPRVGGQDQKDSPVAIPMSSGDTEDPGVASGYVSSADLVFTPNSGASSVSLVPSLGLPSDQTPSLCPGLASGPPGAPGPVKSGFEGYVELPPIEGRSPRSPRNNPVPPEAKSPVLNPGERPADVSPTSPQPEGLLVLQQVGDYCFLPGLGPGPLSLRSKPSSPGPGPEIKNLDQAFQVKKPPGQAVPQVPVIQLFKALKQQDYLSLPPWEVNKPGEVCRAKRAPVKQTLNFDLLKLAGDVESNPGPMVSVIKPEMKIKLCMRGTVNGHNFVIEGEGKGNPYEGTQILDLNVTEGAPLPFAYDILTTVFQYGNRAFTKYPADIQDYFKQTFPEGYHWERSMTYEDQGICTATSNISMRGDCFFYDIRFDGTNFPPNGPVMQKKTLKWEPSTEKMYVEDGVLKGDVNMRLLLEGGGHYRCDFKTTYKAKKEVRLPDAHKIDHRIEILKHDKDYNKVKLYENAVARYSMLPSQAK

SEQ ID NO: 189 - protein, 1599 aa, Homo sapiens
MIIVAHVLLILLGATEILQADLLPDEKISLLPPVNFTIKVTGLAQVLLQWKPNPDQEQRNVNLEYQVKINAPKEDDYETRITESKCVTILHKGFSASVRTILQNDHSLLASSWASAELHAPPGSPGTSIVNLTCTTNTTEDNYSRLRSYQVSLHCTWLVGTDAPEDTQYFLYYRYGSWTEECQEYSKDTLGRNIACWFPRTFILSKGRDWLAVLVNGSSKHSAIRPFDQLFALHAIDQINPPLNVTAEIEGTRLSIQWEKPVSAFPIHCFDYEVKIHNTRNGYLQIEKLMTNAFISIIDDLSKYDVQVRAAVSSMCREAGLWSEWSQPIYVGNDEHKPLREWFVIVIMATICFILLILSLICKICHLWIKLFPPIPAPKSNIKDLFVTTNYEKAGSSETEIEVICYIEKPGVETLEDSVFRAKRAPVKQTLNFDLLKLAGDVESNPGPMVLAQGLLSMALLALCWERSLAGAEETIPLQTLRCYNDYTSHITCRWADTQDAQRLVNVTLIRRVNEDLLEPVSCDLSDDMPWSACPHPRCVPRRCVIPCQSFVVTDVDYFSFQPDRPLGTRLTVTLTQHVQPPEPRDLQISTDQDHFLLTWSVALGSPQSHWLSPGDLEFEVVYKRLQDSWEDAAILLSNTSQATLGPEHLMPSSTYVARVRTRLAPGSRLSGRPSKWSPEVCWDSQPGDEAQPQNLECFFDGAAVLSCSWEVRKEVASSVSFGLFYKPSPDAGEEECSPVLREGLGSLHTRHHCQIPVPDPATHGQYIVSVQPRRAEKHIKSSVNIQMAPPSLNVTKDGDSYSLRWETMKMRYEHIDHTFEIQYRKDTATWKDSKTETLQNAHSMALPALEPSTRYWARVRVRTSRTGYNGIWSEWSEARSWDTESVLPMWVLALIVIFLTIAVLLALRFCGIYGYRLRRKWEEKIPNPSKSHLFQNGSAELWPPGSMSAFTSGSPPHQGPWGSRFPELEGVFPVGFGDSEVSPLTIEDPKHVCDPPSGPDTTPAASDLPTEQPPSPQPGPPAASHTPEKQASSFDFNGPYLGPPHSRSLPDILGQPEPPQEGGSQKSPPPGSLEYLCLPAGGQVQLVPLAQAMGPGQAVEVERRPSQGAAGSPSLESGGGPAPPALGPRVGGQDQKDSPVAIPMSSGDTEDPGVASGYVSSADLVFTPNSGASSVSLVPSLGLPSDQTPSLCPGLASGPPGAPGPVKSGFEGYVELPPIEGRSPRSPRNNPVPPEAKSPVLNPGERPADVSPTSPQPEGLLVLQQVGDYCFLPGLGPGPLSLRSKPSSPGPGPEIKNLDQAFQVKKPPGQAVPQVPVIQLFKALKQQDYLSLPPWEVNKPGEVCRAKRAPVKQTLNFDLLKLAGDVESNPGPMVSVIKPEMKIKLCMRGTVNGHNFVIEGEGKGNPYEGTQILDLNVTEGAPLPFAYDILTTVFQYGNRAFTKYPADIQDYFKQTFPEGYHWERSMTYEDQGICTATSNISMRGDCFFYDIRFDGTNFPPNGPVMQKKTLKWEPSTEKMYVEDGVLKGDVNMRLLLEGGGHYRCDFKTTYKAKKEVRLPDAHKIDHRIEILKHDKDYNKVKLYENAVARYSMLPSQAK

SEQ ID NO: 190 - protein, 120 aa, Homo sapiens
EVQLVQSGAEVKKPGASVKVSCKVSGNTLTDLSMHWVRQAPGKGLEWMGGFDPEDGEKIYAQKFQGRVTMTEDTSTDTAYMELSSLRSEDTAVYYCATGLFYYYYGMDVWGQGTLVTVSS

SEQ ID NO: 191 - protein, 120 aa, Homo sapiens
EVQLVQSGAEVKKPGASVKVSCKVSGNTLTDLSMHWVRQAPGKGLEWMGGFDPEDGEKIYAQKFQGRVTMTEDTSTDTAYMELSSLRSEDTAVYYCATGLFYYYYGMDVWGQGTMVTVSS

SEQ ID NO: 192 - protein, 120 aa, Homo sapiens
EVQLVQSGAEVKKPGASVKVSCKVSGYTLTDLSMHWVRQAPGKGLEWMGGFDPEDGEKIYAQKFQGRVTMTEDTSTDTAYMELSSLRSEDTAVYYCATGLFYYYYGMDVWGQGTTVTVSS

SEQ ID NO: 193 - protein, 120 aa, Homo sapiens
EVQLVQSGAEVKKPGASVKVSCKVSGYTLTDLSMHWVRQAPGKGLEWMGGFDPEDGERIYAQKFQDRVTMTEDTSTDTAYMELSSLRSEDTAVYYCATGLFYYYYGMDVWGQGTTVTVSS

SEQ ID NO: 194 - protein, 120 aa, Homo sapiens
EVQLVQSGAEVKKPGASVKVSCKVSGYTLTDLSMHWVRQAPGKGLEWMGGFDPEDGETIYAQKFQGRVTVTEDTSTDTAYMELSSLRSEDTAVYYCATGLFYYYYGMDVWGQGTTVTVSS

SEQ ID NO: 195 - protein, 120 aa, Homo sapiens
EVQLQQSGAEVKKPGASVKVSCKVSGYTLTDLSMHWVRQAPGKGLEWMGGFDPEDGETIYAQKFQGRVTMTEDTSTDTAYMELSSLRSEDTAVYYCATGLFYYYYGMDVWGQGTLVTVSS

SEQ ID NO: 196 - protein, 120 aa, Homo sapiens
EVQLVQSGAEVKKPGASVKVSCKVSGYTLTDLSMHWVRQAPGKGLEWMGGLDPEDGETIYAQKFQGRVTMTEDTSTDTAYMELSSLRSEDTAVYYCATGLFYYYYGMDVWGQGTTVTVSS

SEQ ID NO: 197 - protein, 120 aa, Homo sapiens
EVQLVQSGAEVKKPGASVKVSCKVSGYTLTDLSMHWVRQAPGKGLEWMGGLDPEDGETIYAQKFQGRVTMTEDTSTDTAYMELSSLRSEDTAVYYCATGLFYYYYGMDVWGQGTLVTVSS

SEQ ID NO: 198 - protein, 120 aa, Homo sapiens
EVQLVQSGAEVKKPGASVKVSCKVSGYTLTDLSMHWVRQAPGKGLEWMGGSDPEDGETIYAQKFQGRVTMTEDTSTDTAYMELSSLRSEDTAVYYCATGLFYYYYGMDVWGQGTTVTVSS

SEQ ID NO: 199 - protein, 120 aa, Homo sapiens
EVQLVQSGAEVKKPGASVKVSCKVSGYTLTDLSMHWVRQAPGKGLEWMGGSDPEDGETIYAQKFQGRVTMTEDISTDTAYMELSSLRSEDTAVYYCATGLFYYYYGMDVWGQGTTVTVSS

SEQ ID NO: 200 - protein, 120 aa, Homo sapiens
EVQLVQSGAEVKKPGASVKVSCKASGYPLSDVALHWVRQAPGKGLEWMGGFDPEDGERIYAQKFQGRVTMTEDTSTDTAYMELSSLRSEDTAVYYCATGLFYYYYGMDVWGQGTMVTVSS

SEQ ID NO: 201 - protein, 120 aa, Homo sapiens
EVQLVQSGAEVKKPGASVKVSCKVSGYPLSDFAMHWVRQAPGKGLEWMGGFDPEDGERIYAQKFQGRVTMTEDTSTDTAYMELSSLRSEDTAVYYCATGLFYYYYGMDVWGQGTMVTVSS

SEQ ID NO: 202 - protein, 120 aa, Homo sapiens
EVQLVQSGAEVKKPGASVKVSCAVSGFGLNDLALHWVRQAPGKGLEWMGGFDPEDGERIYAQKFQGRVTMTEDTSTDTAYMELSSLRSEDTAVYYCATGLFYYYYGMDVWGQGTMVTVSS

SEQ ID NO: 203 - protein, 120 aa, Homo sapiens
EVQLVQSGAEVKKPGASVKVSCEVSGYPLSDYAMHWVRQAPGKGLEWMGGFDPEDGERIYAQKFQGRVTMTEDTSTDTAYMELSSLRSEDTAVYYCATGLFYYYYGMDVWGQGTMVTVSS

SEQ ID NO: 204 - protein, 120 aa, Homo sapiens
EVQLVQSGAEVKKPGASVKVSCEVSGYPLSDFAMHWVRQAPGKGLEWMGGFDPEDGERIYAQKFQGRVTMTEDTSTDTAYMELSSLRSEDTAVYYCATGLFYYYYGMDVWGQGTMVTVSS

SEQ ID NO: 205 - protein, 120 aa, Homo sapiens
EVQLVQSGAEVKKPGASVKVSCKVSGYTLTDLSMHWVRQAPGKGLEWMGGFDPEDGERIYAQKFQGRVTMTEDTSTDTAYMELSSLRSEDTAVYYCATGEFYYYYGMDVWGQGTMVTVSS

SEQ ID NO: 206 - protein, 120 aa, Homo sapiens
EVQLVQSGAEVKKPGASVKVSCKVSGYTLTDLSMHWVRQAPGKGLEWMGGFDPEDGERIYAQKFQGRVTMTEDTSTDTAYMELSSLRSEDTAVYYCATGEFYWMYGMDVWGQGTMVTVSS

SEQ ID NO: 207 - protein, 120 aa, Homo sapiens
EVQLVQSGAEVKKPGASVKVSCKVSGYTLTDLSMHWVRQAPGKGLEWMGGFDPEDGERIYAQKFQGRVTMTEDTSTDTAYMELSSLRSEDTAVYYCASGEFYYYYGMDVWGQGTMVTVSS

SEQ ID NO: 208 - protein, 120 aa, Homo sapiens
EVQLVQSGAEVKKPGASVKVSCTVSGFPISDFAMHWVRQAPGKGLEWMGGFDPEDGERIYAQKFQGRVTMTEDTSTDTAYMELSSLRSEDTAVYYCATGLFYYYYGMDVWGQGTMVTVSS

SEQ ID NO: 209 - protein, 120 aa, Homo sapiens
EVQLVQSGAEVKKPGASVKVSCAVSGFPLTDFALHWVRQAPGKGLEWMGGFDPEDGERIYAQKFQGRVTMTEDTSTDTAYMELSSLRSEDTAVYYCATGLFYYYYGMDVWGQGTMVTVSS

SEQ ID NO: 210 - protein, 298 aa, Homo sapiens
EKSDLRTVAPASSLNVRFDSRTMNLSWDCQENTTFSKCFLTDKKNRVVEPRLSNNECSCTFREICLHEGVTFEVHVNTSQRGFQQKLLYPNSGREGTAAQNFSCFIYNADLMNCTWARGPTAPRDVQYFLYIRNSKRRREIRCPYYIQDSGTHVGCHLDNLSGLTSRNYFLVNGTSREIGIQFFDSLLDTKKIERFNPPSNVTVRCNTTHCLVRWKQPRTYQKLSYLDFQYQLDVHRKNTQPGTENLLINVSGDLENRYNFPSSEPRAKHSVKIRAADVRILNWSSWSEAIEFGSDDG

SEQ ID NO: 211 - protein, 427 aa, Homo sapiens
WERSLAGAEETIPLQTLRCYNDYTSHITCRWADTQDAQRLVNVTLIRRVNEDLLEPVSCDLSDDMPWSACPHPRCVPRRCVIPCQSFVVTDVDYFSFQPDRPLGTRLTVTLTQHVQPPEPRDLQISTDQDHFLLTWSVALGSPQSHWLSPGDLEFEVVYKRLQDSWEDAAILLSNTSQATLGPEHLMPSSTYVARVRTRLAPGSRLSGRPSKWSPEVCWDSQPGDEAQPQNLECFFDGAAVLSCSWEVRKEVASSVSFGLFYKPSPDAGEEECSPVLREGLGSLHTRHHCQIPVPDPATHGQYIVSVQPRRAEKHIKSSVNIQMAPPSLNVTKDGDSYSLRWETMKMRYEHIDHTFEIQYRKDTATWKDSKTETLQNAHSMALPALEPSTRYWARVRVRTSRTGYNGIWSEWSEARSWDTESVLPMW